European Patent Application EP 4 579 240 A1, published July 2, 2025. Title: Cf48肾损伤生物标志物及在肾损伤治疗药物中的用途. Applicant: 广州市康润生物科技有限公司. Application CN 2022106143889, filed June 1, 2022. The sequence listing filed with the application follows.

SEQUENCE LISTING (1 sequence)

SEQ ID NO: 1 - DNA, 289 bp, Homo sapiens
  source 1..289: mol_type = genomic DNA
atggcccccccgcccgcgtgccggtccccgatgtcaccgccgccgccgccgctgctgctgctgctgctgagtctggcgctgctgggcgcccgggcccgcgccgagcccgccgggagtgccgtccccgcgcagagccgcccatgcgtggactgccacgccttcgagttcatgcagcgcgccctgcaggacctgcggaagacagcctgcagcctggacgcgcggacggagaccctactgctgcaggcagagcgccgtgccctgtgtgcctgctggccagcggggcactgag